European Patent Application EP 4 159 846 A1, published April 5, 2023. Title: Low immunogenic cells. Applicant: Healios K.K. The sequence listing filed with the application follows.

SEQUENCE LISTING (24 sequences)

SEQ ID NO: 1 - DNA, 23 bp, Artificial Sequence
  crRNA
acagcgacgccgcgagccagagg

SEQ ID NO: 2 - DNA, 23 bp, Artificial Sequence
  crRNA
cctcctccgcgggtatgaccagg

SEQ ID NO: 3 - DNA, 23 bp, Artificial Sequence
  crRNA
agcgacgccgcgagtccaagagg

SEQ ID NO: 4 - DNA, 20 bp, Artificial Sequence
  primer
aatcagtgtcgtcgcggtcg

SEQ ID NO: 5 - DNA, 21 bp, Artificial Sequence
  primer
agtctgtgagtgggccttcac

SEQ ID NO: 6 - DNA, 25 bp, Artificial Sequence
  primer
gagacacagatctccaagaccaaca

SEQ ID NO: 7 - DNA, 23 bp, Artificial Sequence
  primer
cctgagaggaaaagtcacggttc

SEQ ID NO: 8 - DNA, 20 bp, Artificial Sequence
  primer
agggaaacggcctctgcgga

SEQ ID NO: 9 - DNA, 20 bp, Artificial Sequence
  primer
tctgtgcctggcgcttgtac

SEQ ID NO: 10 - DNA, 23 bp, Artificial Sequence
  crRNA
tgagaccgttcgcttcctgctgg

SEQ ID NO: 11 - DNA, 23 bp, Artificial Sequence
  primer
atacccactcatgacgtgacctg

SEQ ID NO: 12 - DNA, 21 bp, Artificial Sequence
  primer
cagccgcatctcaaagacaag

SEQ ID NO: 13 - DNA, 250 bp, Artificial Sequence
  3'ITR
ccctagaaagataatcatattgtgacgtacgttaaagataatcatgcgtaaaattgacgcatgtgttttatcggtctgtatatcgaggtttatttattaatttgaatagatattaagttttattatatttacacttacatactaataataaattcaacaaacaatttatttatgtttatttatttattaaaaaaaaacaaaaactcaaaatttcttctataaagtaacaaaacttttaaacattctctct

SEQ ID NO: 14 - DNA, 307 bp, Artificial Sequence
  5'ITR
tatctataacaagaaaatatatatataataagttatcacgtaagtagaacatgaaataacaatataattatcgtatgagttaaatcttaaaagtcacgtaaaagataatcatgcgtcattttgactcacgcggtcgttatagttcaaaatcagtgacacttaccgcattgacaagcacgcctcacgggagctccaagcggcgactgagatgtcctaaatgcacagcgacggattcgcgctatttagaaagagagagcaatatttcaagaatgcatgcgtcaattttacgcagactatctttctaggg

SEQ ID NO: 15 - DNA, 1758 bp, Homo sapiens
atgaggatatttgctgtctttatattcatgacctactggcatttgctgaacgcatttactgtcacggttcccaaggacctatatgtggtagagtatggtagcaatatgacaattgaatgcaaattcccagtagaaaaacaattagacctggctgcactaattgtctattgggaaatggaggataagaacattattcaatttgtgcatggagaggaagacctgaaggttcagcatagtagctacagacagagggcccggctgttgaaggaccagctctccctgggaaatgctgcacttcagatcacagatgtgaaattgcaggatgcaggggtgtaccgctgcatgatcagctatggtggtgccgactacaagcgaattactgtgaaagtcaatgccccatacaacaaaatcaaccaaagaattttggttgtggatccagtcacctctgaacatgaactgacatgtcaggctgagggctaccccaaggccgaagtcatctggacaagcagtgaccatcaagtcctgagtggtaagaccaccaccaccaattccaagagagaggagaagcttttcaatgtgaccagcacactgagaatcaacacaacaactaatgagattttctactgcacttttaggagattagatcctgaggaaaaccatacagctgaattggtcatcccagaactacctctggcacatcctccaaatgaaaggactcacttggtaattctgggagccatcttattatgccttggtgtagcactgacattcatcttccgtttaagaaaagggagaatgatggatgtgaaaaaatgtggcatccaagatacaaactcaaagaagcaaagtgatacacatttggaggagacgggaagcggagctactaacttcagcctgctgaagcaggcaggagacgtggaggagaaccctgggcccatgatcttcctcctgctaatgttgagcctggaattgcagcttcaccagatagcagctttattcacagtgacagtccctaaggaactgtacataatagagcatggcagcaatgtgaccctggaatgcaactttgacactggaagtcatgtgaaccttggagcaataacagccagtttgcaaaaggtggaaaatgatacatccccacaccgtgaaagagccactttgctggaggagcagctgcccctagggaaggcctcgttccacatacctcaagtccaagtgagggacgaaggacagtaccaatgcataatcatctatggggtcgcctgggactacaagtacctgactctgaaagtcaaagcttcctacaggaaaataaacactcacatcctaaaggttccagaaacagatgaggtagagctcacctgccaggctacaggttatcctctggcagaagtatcctggccaaacgtcagcgttcctgccaacaccagccactccaggacccctgaaggcctctaccaggtcaccagtgttctgcgcctaaagccaccccctggcagaaacttcagctgtgtgttctggaatactcacgtgagggaacttactttggccagcattgaccttcaaagtcagatggaacccaggacccatccaacttggctgcttcacattttcatccccttctgcatcattgctttcattttcatagccacagtgatagccctaagaaaacaactctgtcaaaagctgtattcttcaaaagacacaacaaaaagacctgtcaccacaacaaagagggaagtgaacagtgctatctga

SEQ ID NO: 16 - DNA, 1017 bp, Homo sapiens
atggtggtcatggcgccccgaaccctcttcctgctactctcgggggccctgaccctgaccgagacctgggcgggctcccactccatgaggtatttcagcgccgccgtgtcccggcccagccgcggggagccccgcttcatcgccatgggctacgtggacgacacgcagttcgtgcggttcgacagcgactcggcgtgtccgaggatggagccgcgggcgccgtgggtggagcgggaggggccagagtattgggaagaggagacacggaacaccaaggcccacgcacagactgacagaatgaacctgcagaccctgcgcggctactacaaccagagcgaggccagttctcataccctccagtggatgattggctgcgacctggggtccgacggacgcctcctccgcgggtatgaacagtatgcctacgatggcaaggattacctcgccctgaacgaggacctgcgctcctggaccgcagcggacactgcggctcagatctccaagcgcaagtgtgaggcggccaatgtggctgaacaaaggagagcctacctggagggcacgtgcgtggagtggctccacagatacctggagaacgggaaggagatgctgcagcgcgcggacccccccaagacacacgtgacccaccaccctgtctttgactatgaggccaccctgaggtgctgggccctgggcttctaccctgcggagatcatactgacctggcagcgggatggggaggaccagacccaggacgtggagctcgtggagaccaagcctgcaggggatggaaccttccagaagtgggcagctgtggtggtgccttctggagaggagcagagatacacgtgccatgtgcagcatgaggggctgccggagcccctcatgctgagatggaagcagtcttccctgcccaccatccccatcatgggtatcgttgctggtctggttgtccttgcagctgtagtcactggagctgcggtcgctgctgtgctgtggaggaagaagagctcagattga

SEQ ID NO: 17 - DNA, 360 bp, Homo sapiens
atgtctcgctccgtggccttagctgtgctcgcgctactctctctttctggcctggaggctatccagcgtactccaaagattcaggtttactcacgtcatccagcagagaatggaaagtcaaatttcctgaattgctatgtgtctgggtttcatccatccgacattgaagttgacttactgaagaatggagagagaattgaaaaagtggagcattcagacttgtctttcagcaaggactggtctttctatctcttgtactacactgaattcacccccactgaaaaagatgagtatgcctgccgtgtgaaccatgtgactttgtcacagcccaagatagttaagtgggatcgagacatgtaa

SEQ ID NO: 18 - DNA, 1785 bp, Artificial Sequence
  PBase
atgggaagctccctggacgatgaacatatcctctccgctctgctccaaagcgatgacgaactggtgggcgaggattccgactctgagatttctgaccatgtcagcgaggacgatgtgcagtccgatactgaagaggcatttatcgacgaggtgcatgaagtccagcccacttcctctggaagcgaaatcctggacgagcagaatgtcatcgaacagcctggctcctctctcgcttccaacagaatcctgaccctccctcagaggacaatcagaggcaagaacaagcattgctggtctacaagcaaatccaccaggagaagccgggtgtctgccctcaatatcgtcagaagccaaaggggacccacccggatgtgtaggaacatttacgatcctctgctctgcttcaagctgtttttcactgacgagatcatttctgaaattgtgaagtggacaaacgccgaaatctctctcaagagaagggaaagcatgacaggggctacattcagggacacaaatgaggatgaaatttacgccttctttggcattctggtgatgacagcagtcagaaaagataatcacatgagcacagatgatctcttcgacagatccctgagcatggtgtatgtctctgtgatgtccagagatcggttcgattttctcattagatgcctgcggatggacgataaatccatcaggcccactctcagagagaatgatgtgttcacccctgtgcggaagatttgggatctgttcatccaccagtgcattcaaaattacacccccggcgctcatctcacaatcgacgaacaactcctgggatttcggggcagatgtcccttcagaatgtatattcctaataagccaagcaagtacgggatcaaaattctgatgatgtgtgactctggaaccaagtatatgattaacggaatgccttatctcggcagagggacccaaactaacggcgtgccactcggcgaatactatgtcaaagagctgtccaaacctgtccacggaagctgtagaaatatcacctgcgataactggtttacatccattcccctcgccaagaacctgctccaagaaccttacaagctgaccattgtcggcactgtcaggtccaacaagagggagattccagaagtgctcaagaactccagaagcaggccagtcggcacatccatgttctgtttcgacggaccactgactctcgtgtcttacaagcccaaacctgctaagatggtctatctgctcagctcctgtgatgaggacgcctctattaacgagagcaccggcaagccacaaatggtgatgtactataaccagaccaaggggggagtcgatactctcgaccagatgtgttccgtgatgacatgctccagaaagactaatcggtggcctatggctctcctgtatggcatgattaacattgcctgtatcaacagcttcatcatttatagccacaacgtgtcctctaagggagaaaaggtccaaagcagaaagaaattcatgcggaacctgtatatgagcctcacctcctcttttatgcggaagaggctggaggcacctactctcaaaagatacctgagggataacatcagcaacattctccctaatgaggtccccggaacatccgacgattctactgaggaacctgtgatgaagaaacggacctattgcacatactgtcctagcaagatcagaaggaaggcaaatgcttcctgcaagaaatgtaagaaggtcatttgtagagaacataacattgatatgtgtcagagctgcttctaa

SEQ ID NO: 19 - DNA, 1554 bp, Homo sapiens
atggccagcagaatcctgtggcacgagatgtggcatgaaggcctggaagaggccagcaggctgtacttcggcgagagaaacgtgaagggcatgttcgaggtgctggaacccctgcacgccatgatggaaagaggccctcagacactgaaagagacaagcttcaaccaggcctacggccgggatctgatggaagcccaagagtggtgccggaagtacatgaagtccggcaatgtgaaggacctgctgcaggcctgggacctgtactaccacgtgttcagacggatcagcaagctcgagtacagcggcggaggatctctggaaggcgtccaggtggaaacaatctctcctggcgacggccggacattccctaaaaggggccagacatgcgtggtgcactacaccggcatgctggaagatggcaagaagttcgacagcagccgggacagaaacaagcccttcaagttcatgctgggcaagcaagaagtgatcagaggctgggaagagggcgtcgcccagatgtctgttggacagagagccaagctgacaatcagccccgattacgcctatggcgccacaggacaccctggcatcattcctccacatgccacactggtgttcgacgtggaactgctgaagctggaatctggcggaggtggaagcggaggcggaggttctggtggtggtggatctggcgttgacggctttggagatgtgggcgccctggaaagcctgagaggaaatgccgatctggcctacatcctgagcatggaaccttgcggccactgcctgattatcaacaacgtgaacttctgcagagagagcggcctgagaaccagaaccggcagcaacatcgactgcgagaagctgcggagaagattcagcagcctgcacttcatggtggaagtgaagggcgacctgaccgccaagaaaatggtgctggctctgctggaactggcccagcaagatcatggcgctctggattgctgcgtggtcgtgatcctgtctcatggctgtcaggccagccatctgcaattccctggcgccgtgtatggcaccgatggctgtcctgtgtccgtggaaaagatcgtgaacatcttcaacggcaccagctgtcctagcctcggcggaaagcccaagctgttcttcatccaagcctgtggcggcgagcagaaggatcacggatttgaggtggccagcacaagccccgaggatgagtctcctggaagcaaccctgagcctgacgccacacctttccaagagggactgagaaccttcgaccagctggacgctatcagctccctgcctacacctagcgacatcttcgtgtcctacagcacattccccggctttgtgtcttggcgggatcccaagtctggctcttggtacgtggaaaccctggacgatatcttcgagcagtgggcccatagcgaggacctgcaatctctgctgctgagagtggccaatgccgtgtccgtgaagggaatctacaagcagatgcctggctgcttcaacttcctgcggaagaagctgtttttcaagaccagcgccagctga

SEQ ID NO: 20 - DNA, 20 bp, Artificial Sequence
  primer
gaactgctgaagctggaatc

SEQ ID NO: 21 - DNA, 22 bp, Artificial Sequence
  primer
catttcctctcaggctttccag

SEQ ID NO: 22 - DNA, 28 bp, Artificial Sequence
  probe
atctggcgttgacggctttggagatgtg

SEQ ID NO: 23 - DNA, 1706 bp, Artificial Sequence
  IRES-Puro-hGHpolyA
cgcccctctccctcccccccccctaacgttactggccgaagccgcttggaataaggccggtgtgcgtttgtctatatgtgattttccaccatattgccgtcttttggcaatgtgagggcccggaaacctggccctgtcttcttgacgagcattcctaggggtctttcccctctcgccaaaggaatgcaaggtctgttgaatgtcgtgaaggaagcagttcctctggaagcttcttgaagacaaacaacgtctgtagcgaccctttgcaggcagcggaaccccccacctggcgacaggtgcctctgcggccaaaagccacgtgtataagatacacctgcaaaggcggcacaaccccagtgccacgttgtgagttggatagttgtggaaagagtcaaatggctctcctcaagcgtattcaacaaggggctgaaggatgcccagaaggtaccccattgtatgggatctgatctggggcctcggtgcacatgctttacatgtgtttagtcgaggttaaaaaaacgtctaggccccccgaaccacggggacgtggttttcctttgaaaaacacgatgataatatggccacaaccatgaccgaatataaacctacggttagattggcgacaagggacgacgtgcctagagctgtacgcacactggcagccgcatttgcggactacccggcaacacgacacaccgtggaccctgatcgccacatagagcgggtcactgaactccaggaattgtttctcacccgagtaggccttgacattggcaaggtatgggtcgcggacgacggtgccgccgttgctgtctggactaccccggaaagcgtagaagctggagctgtattcgcagagatcggtccaaggatggcagagctttctggctccagacttgccgcccaacaacagatggaaggacttctggcgccccataggccgaaagagcctgcgtggtttttggctacagttggcgtttccccagatcatcaaggtaaagggctcggatctgccgtggtgcttcctggggttgaggcagctgagagggccggtgttcctgcgttccttgagacatccgctcctcgcaacttgcctttctatgaaaggctgggttttactgttacggccgatgtagaagtgccagaaggaccacgcacctggtgcatgactagaaagcctggggcatgaataacttcgtatagcatacattatacgaagttatctgcccgggtggcatccctgtgacccctccccagtgcctctcctggccctggaagttgccactccagtgcccaccagccttgtcctaataaaattaagttgcatcattttgtctgactaggtgtccttctataatattatggggtggaggggggtggtatggagcaaggggcaagttgggaagacaacctgtagggcctgcggggtctattgggaaccaagctggagtgcagtggcacaatcttggctcactgcaatctccgcctcctgggttcaagcgattctcctgcctcagcctcccgagttgttgggattccaggcatgcatgaccaggctcagctaatttttgtttttttggtagagacggggtttcaccatattggccaggctggtctccaactcctaatctcaggtgatctacccaccttggcctcccaaattgctgggattacaggcgtgaaccactgctcccttccctgtcctt

SEQ ID NO: 24 - DNA, 2144 bp, Artificial Sequence
  IRES-Hygro-hGHpolyA
cgcccctctccctcccccccccctaacgttactggccgaagccgcttggaataaggccggtgtgcgtttgtctatatgtgattttccaccatattgccgtcttttggcaatgtgagggcccggaaacctggccctgtcttcttgacgagcattcctaggggtctttcccctctcgccaaaggaatgcaaggtctgttgaatgtcgtgaaggaagcagttcctctggaagcttcttgaagacaaacaacgtctgtagcgaccctttgcaggcagcggaaccccccacctggcgacaggtgcctctgcggccaaaagccacgtgtataagatacacctgcaaaggcggcacaaccccagtgccacgttgtgagttggatagttgtggaaagagtcaaatggctctcctcaagcgtattcaacaaggggctgaaggatgcccagaaggtaccccattgtatgggatctgatctggggcctcggtgcacatgctttacatgtgtttagtcgaggttaaaaaaacgtctaggccccccgaaccacggggacgtggttttcctttgaaaaacacgatgataatatggccacaaccatgaaaaagcctgaactcaccgcgacgtctgtcgagaagtttctgatcgaaaagttcgacagcgtctccgacctgatgcagctctcggagggcgaagaatctcgtgctttcagcttcgatgtaggagggcgtggatatgtcctgcgggtaaatagctgcgccgatggtttctacaaagatcgttatgtttatcggcactttgcatcggccgcgctcccgattccggaagtgcttgacattggggaattcagcgagagcctgacctattgcatctcccgccgtgcacagggtgtcacgttgcaagacctgcctgaaaccgaactgcccgctgttctgcagccggtcgcggaggccatggatgcgatcgctgcggccgatcttagccagacgagcgggttcggcccattcggaccgcaaggaatcggtcaatacactacatggcgtgatttcatatgcgcgattgctgatccccatgtgtatcactggcaaactgtgatggacgacaccgtcagtgcgtccgtcgcgcaggctctcgatgagctgatgctttgggccgaggactgccccgaagtccggcacctcgtgcacgcggatttcggctccaacaatgtcctgacggacaatggccgcataacagcggtcattgactggagcgaggcgatgttcggggattcccaatacgaggtcgccaacatcttcttctggaggccgtggttggcttgtatggagcagcagacgcgctacttcgagcggaggcatccggagcttgcaggatcgccgcggctccgggcgtatatgctccgcattggtcttgaccaactctatcagagcttggttgacggcaatttcgatgatgcagcttgggcgcagggtcgatgcgacgcaatcgtccgatccggagccgggactgtcgggcgtacacaaatcgcccgcagaagcgcggccgtctggaccgatggctgtgtagaagtactcgccgatagtggaaaccgacgccccagcactcgtggggatcgggagatgggggaggctaactgaataacttcgtataggataccttatacgaagttatctgcccgggtggcatccctgtgacccctccccagtgcctctcctggccctggaagttgccactccagtgcccaccagccttgtcctaataaaattaagttgcatcattttgtctgactaggtgtccttctataatattatggggtggaggggggtggtatggagcaaggggcaagttgggaagacaacctgtagggcctgcggggtctattgggaaccaagctggagtgcagtggcacaatcttggctcactgcaatctccgcctcctgggttcaagcgattctcctgcctcagcctcccgagttgttgggattccaggcatgcatgaccaggctcagctaatttttgtttttttggtagagacggggtttcaccatattggccaggctggtctccaactcctaatctcaggtgatctacccaccttggcctcccaaattgctgggattacaggcgtgaaccactgctcccttccctgtcctt